European Patent Specification EP 3 821 912 B1, published June 12, 2024. Title: RPGR GENE THERAPY FOR RETINITIS PIGMENTOSA. Applicant: Massachusetts Eye and Ear Infirmary. The sequence listing filed with the application follows.

SEQUENCE LISTING (5 sequences)

SEQ ID NO: 1 - DNA, 3081 bp, Artificial Sequence
  Human RPGRORF15 sequence with 378bp deleted
atgagggagccggaagagctgatgcccgattcgggtgctgtgtttacatttgggaaaagtaaatttgctgaaaataatcccggtaaattctggtttaaaaatgatgtccctgtacatctttcatgtggagatgaacattctgctgttgttaccggaaataataaactttacatgtttggcagtaacaactggggtcagttaggattaggatcaaagtcagccatcagcaagccaacatgtgtcaaagctctaaaacctgaaaaagtgaaattagctgcctgtggaaggaaccacaccctggtgtcaacagaaggaggcaatgtatatgcaactggtggaaataatgaaggacagttggggcttggtgacaccgaagaaagaaacacttttcatgtaattagcttttttacatccgagcataagattaagcagctgtctgctggatctaatacttcagctgccctaactgaggatggaagactttttatgtggggtgacaattccgaagggcaaattggtttaaaaaatgtaagtaatgtctgtgtccctcagcaagtgaccattgggaaacctgtctcctggatctcttgtggatattaccattcagcttttgtaacaacagatggtgagctatatgtgtttggagaacctgagaatgggaagttaggtcttcccaatcagctcctgggcaatcacagaacaccccagctggtgtctgaaattccggagaaggtgatccaagtagcctgtggtggagagcatactgtggttctcacggagaatgctgtgtatacctttgggctgggacaatttggtcagctgggtcttggcacttttctttttgaaacttcagaacccaaagtcattgagaatattagggatcaaacaataagttatatttcttgtggagaaaatcacacagctttgataacagatatcggccttatgtatacttttggagatggtcgccacggaaaattaggacttggactggagaattttaccaatcacttcattcctactttgtgctctaattttttgaggtttatagttaaattggttgcttgtggtggatgtcacatggtagtttttgctgctcctcatcgtggtgtggcaaaagaaattgaattcgatgaaataaatgatacttgcttatctgtggcgacttttctgccgtatagcagtttaacctcaggaaatgtactgcagaggactctatcagcacgtatgcggcgaagagagagggagaggtctccagattctttttcaatgaggagaacactacctccaatagaagggactcttggcctttctgcttgttttctccccaattcagtctttccacgatgttctgagagaaacctccaagagagtgtcttatctgaacaggacctcatgcagccagaggaaccagattatttgctagatgaaatgaccaaagaagcagagatagataattcttcaactgtagaaagccttggagaaactactgatatcttaaacatgacacacatcatgagcctgaattccaatgaaaagtcattaaaattatcaccagttcagaaacaaaagaaacaacaaacaattggggaactgacgcaggatacagctcttactgaaaacgatgatagtgatgaatatgaagaaatgtcagaaatgaaagaagggaaagcatgtaaacaacatgtgtcacaagggattttcatgacgcagccagctacgactatcgaagcattttcagatgaggaagtagagatcccagaggagaaggaaggagcagaggattcaaaaggaaatggaatagaggagcaagaggtagaagcaaatgaggaaaatgtgaaggtgcatggaggaagaaaggagaaaacagagatcctatcagatgaccttacagacaaagcagaggtgagtgaaggcaaggcaaaatcagtgggagaagcagaggatgggcctgaaggtagaggggatggaacctgtgaggaaggtagttcaggagcagaacactggcaagatgaggagagggagaagggggagaaagacaagggtagaggagaaatggagaggccaggagagggagagaaggaactagcagagaaggaagaatggaagaagagggatggggaagagcaggagcaaaaggagagggagcagggccatcagaaggaaagaaaccaagagatggaggagggaggggaggaggagcatggagaaggagaagaagaggagggagacagagaagaggaagaagagaaggagggagaagggaaagaggaaggagaaggggaagaagtggagggagaacgtgaaaaggaggaaggagagaggaaaaaggaggaaagagcggggaaggaggagaaaggagaggaagaaggagaccaaggagagggggaagaggaggaaacagaggggagaggggaggaaaaagaggagggaggggaagtagagggaggggaagtagaggaggggaaaggagagagggaagaggaagaggaggagggtgagggggaagaggaggaaggggagggggaagaggaggaaggggagggggaagaggaggaaggagaagggaaaggggaggaagaaggggagggggaagaggaggaaggggaagaagaaggggaggaagaaggagagggagaggaagaaggggagggagaaggggaggaagaagaggaaggggaagtggaaggggaggtggaaggggaggaaggagagggggaaggagaggaagaggaaggagaggaggaaggagaagaaagggaaaaggagggggaaggagaagaaaacaggaggaacagagaagaggaggaggaagaagaggggaagtatcaggagacaggcgaagaagagaatgaaaggcaggatggagaggagtacaaaaaagtgagcaaaataaaaggatctgtgaaatatggcaaacataaaacatatcaaaaaaagtcagttactaacacacagggaaatgggaaagagcagaggtccaaaatgccagtccagtcaaaacgacttttaaaaaatgggccatcaggttccaaaaagttctggaataatatattaccacattacttggaattgaagtaa

SEQ ID NO: 2 - protein, 1026 aa, Artificial Sequence
  Human RPGRORF15 sequence with 126 amino acids deleted
MREPEELMPDSGAVFTFGKSKFAENNPGKFWFKNDVPVHLSCGDEHSAVVTGNNKLYMFGSNNWGQLGLGSKSAISKPTCVKALKPEKVKLAACGRNHTLVSTEGGNVYATGGNNEGQLGLGDTEERNTFHVISFFTSEHKIKQLSAGSNTSAALTEDGRLFMWGDNSEGQIGLKNVSNVCVPQQVTIGKPVSWISCGYYHSAFVTTDGELYVFGEPENGKLGLPNQLLGNHRTPQLVSEIPEKVIQVACGGEHTVVLTENAVYTFGLGQFGQLGLGTFLFETSEPKVIENIRDQTISYISCGENHTALITDIGLMYTFGDGRHGKLGLGLENFTNHFIPTLCSNFLRFIVKLVACGGCHMVVFAAPHRGVAKEIEFDEINDTCLSVATFLPYSSLTSGNVLQRTLSARMRRRERERSPDSFSMRRTLPPIEGTLGLSACFLPNSVFPRCSERNLQESVLSEQDLMQPEEPDYLLDEMTKEAEIDNSSTVESLGETTDILNMTHIMSLNSNEKSLKLSPVQKQKKQQTIGELTQDTALTENDDSDEYEEMSEMKEGKACKQHVSQGIFMTQPATTIEAFSDEEVEIPEEKEGAEDSKGNGIEEQEVEANEENVKVHGGRKEKTEILSDDLTDKAEVSEGKAKSVGEAEDGPEGRGDGTCEEGSSGAEHWQDEEREKGEKDKGRGEMERPGEGEKELAEKEEWKKRDGEEQEQKEREQGHQKERNQEMEEGGEEEHGEGEEEEGDREEEEEKEGEGKEEGEGEEVEGEREKEEGERKKEERAGKEEKGEEEGDQGEGEEEETEGRGEEKEEGGEVEGGEVEEGKGEREEEEEEGEGEEEEGEGEEEEGEGEEEEGEGKGEEEGEGEEEEGEEEGEEEGEGEEEGEGEGEEEEEGEVEGEVEGEEGEGEGEEEEGEEEGEEREKEGEGEENRRNREEEEEEEGKYQETGEEENERQDGEEYKKVSKIKGSVKYGKHKTYQKKSVTNTQGNGKEQRSKMPVQSKRLLKNGPSGSKKFWNNILPHYLELK

SEQ ID NO: 3 - DNA, 3459 bp, Homo sapiens
atgagggagccggaagagctgatgcccgattcgggtgctgtgtttacatttgggaaaagtaaatttgctgaaaataatcccggtaaattctggtttaaaaatgatgtccctgtacatctttcatgtggagatgaacattctgctgttgttaccggaaataataaactttacatgtttggcagtaacaactggggtcagttaggattaggatcaaagtcagccatcagcaagccaacatgtgtcaaagctctaaaacctgaaaaagtgaaattagctgcctgtggaaggaaccacaccctggtgtcaacagaaggaggcaatgtatatgcaactggtggaaataatgaaggacagttggggcttggtgacaccgaagaaagaaacacttttcatgtaattagcttttttacatccgagcataagattaagcagctgtctgctggatctaatacttcagctgccctaactgaggatggaagactttttatgtggggtgacaattccgaagggcaaattggtttaaaaaatgtaagtaatgtctgtgtccctcagcaagtgaccattgggaaacctgtctcctggatctcttgtggatattaccattcagcttttgtaacaacagatggtgagctatatgtgtttggagaacctgagaatgggaagttaggtcttcccaatcagctcctgggcaatcacagaacaccccagctggtgtctgaaattccggagaaggtgatccaagtagcctgtggtggagagcatactgtggttctcacggagaatgctgtgtatacctttgggctgggacaatttggtcagctgggtcttggcacttttctttttgaaacttcagaacccaaagtcattgagaatattagggatcaaacaataagttatatttcttgtggagaaaatcacacagctttgataacagatatcggccttatgtatacttttggagatggtcgccacggaaaattaggacttggactggagaattttaccaatcacttcattcctactttgtgctctaattttttgaggtttatagttaaattggttgcttgtggtggatgtcacatggtagtttttgctgctcctcatcgtggtgtggcaaaagaaattgaattcgatgaaataaatgatacttgcttatctgtggcgacttttctgccgtatagcagtttaacctcaggaaatgtactgcagaggactctatcagcacgtatgcggcgaagagagagggagaggtctccagattctttttcaatgaggagaacactacctccaatagaagggactcttggcctttctgcttgttttctccccaattcagtctttccacgatgttctgagagaaacctccaagagagtgtcttatctgaacaggacctcatgcagccagaggaaccagattatttgctagatgaaatgaccaaagaagcagagatagataattcttcaactgtagaaagccttggagaaactactgatatcttaaacatgacacacatcatgagcctgaattccaatgaaaagtcattaaaattatcaccagttcagaaacaaaagaaacaacaaacaattggggaactgacgcaggatacagctcttactgaaaacgatgatagtgatgaatatgaagaaatgtcagaaatgaaagaagggaaagcatgtaaacaacatgtgtcacaagggattttcatgacgcagccagctacgactatcgaagcattttcagatgaggaagtagagatcccagaggagaaggaaggagcagaggattcaaaaggaaatggaatagaggagcaagaggtagaagcaaatgaggaaaatgtgaaggtgcatggaggaagaaaggagaaaacagagatcctatcagatgaccttacagacaaagcagaggtgagtgaaggcaaggcaaaatcagtgggagaagcagaggatgggcctgaaggtagaggggatggaacctgtgaggaaggtagttcaggagcagaacactggcaagatgaggagagggagaagggggagaaagacaagggtagaggagaaatggagaggccaggagagggagagaaggaactagcagagaaggaagaatggaagaagagggatggggaagagcaggagcaaaaggagagggagcagggccatcagaaggaaagaaaccaagagatggaggagggaggggaggaggagcatggagaaggagaagaagaggagggagacagagaagaggaagaagagaaggagggagaagggaaagaggaaggagaaggggaagaagtggagggagaacgtgaaaaggaggaaggagagaggaaaaaggaggaaagagcggggaaggaggagaaaggagaggaagaaggagaccaaggagagggggaagaggaggaaacagaggggagaggggaggaaaaagaggagggaggggaagtagagggaggggaagtagaggaggggaaaggagagagggaagaggaagaggaggagggtgagggggaagaggaggaaggggagggggaagaggaggaaggggagggggaagaggaggaaggagaagggaaaggggaggaagaaggggaagaaggagaaggggaggaagaaggggaggaaggagaaggggagggggaagaggaggaaggagaaggggagggagaagaggaaggagaaggggagggagaagaggaggaaggagaaggggagggagaagaggaaggagaaggggagggagaagaggaggaaggagaagggaaaggggaggaggaaggagaggaaggagaaggggagggggaagaggaggaaggagaaggggaaggggaggatggagaaggggagggggaagaggaggaaggagaatgggagggggaagaggaggaaggagaaggggagggggaagaggaaggagaaggggaaggggaggaaggagaaggggagggggaagaggaggaaggagaaggggagggggaagaggaggaaggggaagaagaaggggaggaagaaggagagggagaggaagaaggggagggagaaggggaggaagaagaggaaggggaagtggaaggggaggtggaaggggaggaaggagagggggaaggagaggaagaggaaggagaggaggaaggagaagaaagggaaaaggagggggaaggagaagaaaacaggaggaacagagaagaggaggaggaagaagaggggaagtatcaggagacaggcgaagaagagaatgaaaggcaggatggagaggagtacaaaaaagtgagcaaaataaaaggatctgtgaaatatggcaaacataaaacatatcaaaaaaagtcagttactaacacacagggaaatgggaaagagcagaggtccaaaatgccagtccagtcaaaacgacttttaaaaaatgggccatcaggttccaaaaagttctggaataatatattaccacattacttggaattgaagtaa

SEQ ID NO: 4 - protein, 1152 aa, Homo sapiens
MREPEELMPDSGAVFTFGKSKFAENNPGKFWFKNDVPVHLSCGDEHSAVVTGNNKLYMFGSNNWGQLGLGSKSAISKPTCVKALKPEKVKLAACGRNHTLVSTEGGNVYATGGNNEGQLGLGDTEERNTFHVISFFTSEHKIKQLSAGSNTSAALTEDGRLFMWGDNSEGQIGLKNVSNVCVPQQVTIGKPVSWISCGYYHSAFVTTDGELYVFGEPENGKLGLPNQLLGNHRTPQLVSEIPEKVIQVACGGEHTVVLTENAVYTFGLGQFGQLGLGTFLFETSEPKVIENIRDQTISYISCGENHTALITDIGLMYTFGDGRHGKLGLGLENFTNHFIPTLCSNFLRFIVKLVACGGCHMVVFAAPHRGVAKEIEFDEINDTCLSVATFLPYSSLTSGNVLQRTLSARMRRRERERSPDSFSMRRTLPPIEGTLGLSACFLPNSVFPRCSERNLQESVLSEQDLMQPEEPDYLLDEMTKEAEIDNSSTVESLGETTDILNMTHIMSLNSNEKSLKLSPVQKQKKQQTIGELTQDTALTENDDSDEYEEMSEMKEGKACKQHVSQGIFMTQPATTIEAFSDEEVEIPEEKEGAEDSKGNGIEEQEVEANEENVKVHGGRKEKTEILSDDLTDKAEVSEGKAKSVGEAEDGPEGRGDGTCEEGSSGAEHWQDEEREKGEKDKGRGEMERPGEGEKELAEKEEWKKRDGEEQEQKEREQGHQKERNQEMEEGGEEEHGEGEEEEGDREEEEEKEGEGKEEGEGEEVEGEREKEEGERKKEERAGKEEKGEEEGDQGEGEEEETEGRGEEKEEGGEVEGGEVEEGKGEREEEEEEGEGEEEEGEGEEEEGEGEEEEGEGKGEEEGEEGEGEEEGEEGEGEGEEEEGEGEGEEEGEGEGEEEEGEGEGEEEGEGEGEEEEGEGKGEEEGEEGEGEGEEEEGEGEGEDGEGEGEEEEGEWEGEEEEGEGEGEEEGEGEGEEGEGEGEEEEGEGEGEEEEGEEEGEEEGEGEEEGEGEGEEEEEGEVEGEVEGEEGEGEGEEEEGEEEGEEREKEGEGEENRRNREEEEEEEGKYQETGEEENERQDGEEYKKVSKIKGSVKYGKHKTYQKKSVTNTQGNGKEQRSKMPVQSKRLLKNGPSGSKKFWNNILPHYLELK

SEQ ID NO: 5 - DNA, 199 bp, Homo sapiens
gggccccagaagcctggtggttgtttgtccttctcaggggaaaagtgaggcggccccttggaggaaggggccgggcagaatgatctaatcggattccaagcagctcaggggattgtctttttctagcaccttcttgccactcctaagcgtcctccgtgaccccggctgggatttagcctggtgctgtgtcagccccggt